European Patent Specification EP 4 060 030 B1, published September 6, 2023. Title: Novel tetrahydrodipicolinate N-succinyltransferase variant and a method for producing L-valine using the same. Applicant: CJ CheilJedang Corporation. The sequence listing filed with the application follows.

SEQUENCE LISTING (11 sequences)

SEQ ID NO: 1 - protein, 316 aa, Artificial Sequence
  Tetrahydrodipicolinate N-succinyltransferase variant
MSENIRGAQAVGIANIAMDGTILDTWYPEPQIFNPDQWAERYPLKVGTTRLGANELTPRMLQLVKLDQDRLVEQVAVRTVIPDLSQPPVDAHDVYLRLHLLSHRLVRPHEMHMQNTLELLSDVVWTNKGPCLPENFEWVCGALRSRGLIHVYCVDRLPRMVDYVVPPGVRISEAERVRLGAYLAPGTSVLREGFVSFNSGTLGAAKVEGRLSSGVVIGEGSEIGLSSTIQSPRDEQRRRLPLSIGQNCNFGVSSGIIGVSLGDNCDIGNNIVLDGDTPIWFADDEELRTIDSIEGQANWSIKRESGFHEPVARLKA

SEQ ID NO: 2 - DNA, 951 bp, Artificial Sequence
  Tetrahydrodipicolinate N-succinyltransferase variant coding gene
atgagtgaaaacattcgcggagcccaagcagttggaatcgcaaatatcgccatggacgggaccatcctggacacgtggtacccagaaccccaaattttcaacccagatcagtgggctgaacgctacccattgaaagtgggcaccacacgcctcggagcaaacgaactcaccccacggatgctgcagctggtaaaactggaccaagatcgcctcgtcgaacaggtagcagtccgcaccgttatccccgatctgtctcaacctccagtagacgcgcacgatgtttacctgcgcctccacctgctttcccaccgcctggtccgcccccacgaaatgcacatgcaaaacaccttggagctgctgtccgacgtggtgtggacaaacaaaggcccttgccttcctgaaaactttgagtgggtgtgtggtgctctgcggtcccgcggactcatccacgtctactgtgtggaccgtcttccccgcatggtcgactatgtggttccccctggagtccgcatctccgaagcagaacgcgtgcgcctaggtgcataccttgctccgggtacctctgtcctgcgtgaaggtttcgtgtctttcaactccggcaccttgggtgccgcaaaggtggaaggccgcctgagttccggtgtggtcatcggtgaaggttccgagattggactgtcttctactattcagtccccgagagatgaacagcgccgccgtttgccgttgagcatcggccaaaactgcaactttggtgtcagctccggaatcatcggagtcagtctgggagacaattgcgacatcggaaataacattgtcttggatggagatacccccatttggttcgcagacgatgaggagttgcgcactatcgactccatcgaaggccaagcaaattggtcaatcaagcgtgaatccggcttccatgagccagttgcccgcctcaaagcttga

SEQ ID NO: 3 - protein, 316 aa, Artificial Sequence
  Wild-type tetrahydrodipicolinate N-succinyltransferase
MSENIRGAQAVGIANIAMDGTILDTWYPEPQIFNPDQWAERYPLKVGTTRLGANELTPRMLQLVKLDQDRLVEQVAVRTVIPDLSQPPVDAHDVYLRLHLLSHRLVRPHEMHMQNTLELLSDVVWTNKGPCLPENFEWVRGALRSRGLIHVYCVDRLPRMVDYVVPPGVRISEAERVRLGAYLAPGTSVLREGFVSFNSGTLGAAKVEGRLSSGVVIGEGSEIGLSSTIQSPRDEQRRRLPLSIGQNCNFGVSSGIIGVSLGDNCDIGNNIVLDGDTPIWFADDEELRTIDSIEGQANWSIKRESGFHEPVARLKA

SEQ ID NO: 4 - DNA, 951 bp, Artificial Sequence
  Wild-type tetrahydrodipicolinate N-succinyltransferase coding gene
atgagtgaaaacattcgcggagcccaagcagttggaatcgcaaatatcgccatggacgggaccatcctggacacgtggtacccagaaccccaaattttcaacccagatcagtgggctgaacgctacccattgaaagtgggcaccacacgcctcggagcaaacgaactcaccccacggatgctgcagctggtaaaactggaccaagatcgcctcgtcgaacaggtagcagtccgcaccgttatccccgatctgtctcaacctccagtagacgcgcacgatgtttacctgcgcctccacctgctttcccaccgcctggtccgcccccacgaaatgcacatgcaaaacaccttggagctgctgtccgacgtggtgtggacaaacaaaggcccttgccttcctgaaaactttgagtgggtgcgtggtgctctgcggtcccgcggactcatccacgtctactgtgtggaccgtcttccccgcatggtcgactatgtggttccccctggagtccgcatctccgaagcagaacgcgtgcgcctaggtgcataccttgctccgggtacctctgtcctgcgtgaaggtttcgtgtctttcaactccggcaccttgggtgccgcaaaggtggaaggccgcctgagttccggtgtggtcatcggtgaaggttccgagattggactgtcttctactattcagtccccgagagatgaacagcgccgccgtttgccgttgagcatcggccaaaactgcaactttggtgtcagctccggaatcatcggagtcagtctgggagacaattgcgacatcggaaataacattgtcttggatggagatacccccatttggttcgcagacgatgaggagttgcgcactatcgactccatcgaaggccaagcaaattggtcaatcaagcgtgaatccggcttccatgagccagttgcccgcctcaaagcttga

SEQ ID NO: 5 - DNA, 36 bp, Artificial Sequence
  dapD2_1F
tcgagctcggtacccatgagtgaaaacattcgcgga

SEQ ID NO: 6 - DNA, 44 bp, Artificial Sequence
  dapD2_2R
ccgcgggaccgcagagcaccacacacccactcaaagttttcagg

SEQ ID NO: 7 - DNA, 44 bp, Artificial Sequence
  dapD2_3F
cctgaaaactttgagtgggtgtgtggtgctctgcggtcccgcgg

SEQ ID NO: 8 - DNA, 36 bp, Artificial Sequence
  dapD2_4R
ctctagaggatccccccggattcacgcttgattgac

SEQ ID NO: 9 - DNA, 21 bp, Artificial Sequence
  dapD2_5F
atgagtgaaaacattcgcgga

SEQ ID NO: 10 - DNA, 21 bp, Artificial Sequence
  dapD2_6R
ccggattcacgcttgattgac

SEQ ID NO: 11 - DNA, 5803 bp, Artificial Sequence
  pDCM2
gttcgcttgctgtccataaaaccgcccagtctagctatcgccatgtaagcccactgcaagctacctgctttctctttgcgcttgcgttttcccttgtccagatagcccagtagctgacattcatccggggtcagcaccgtttctgcggactggctttctacgtgttccgcttcctttagcagcccttgcgccctgagtgcttgcggcagcgtgaagctagcttttatcgccattcgccattcaggctgcgcaactgttgggaagggcgatcggtgcgggcctcttcgctattacgccagctggcgaaagggggatgtgctgcaaggcgattaagttgggtaacgccagggttttcccagtcacgacgttgtaaaacgacggccagtgaattcgagctcggtacccggggatcctctagagtcgacctgcaggcatgcaagcttggcgtaatcatggtcatagctgtttcctgtgtgaaattgttatccgctcacaattccacacaacatacgagccggaagcataaagtgtaaagcctggggtgcctaatgagtgagctaactcacattaattgcgttgcgctcactgcccgctttccagtcgggaaacctgtcgtgccagctgcattaatgaatcggccaacgcgcggggagaggcggtttgcgtattgggcgctcttccgcttcctcgctcactgactcgctgcgctcggtcgttcggctgcggcgagcggtatcagctcactcaaaggcggtaatacggttatccacagaatcaggggataacgcaggaaagaacatgtgagcaaaaggccagcaaaaggccaggaaccgtaaaaaggccgcgttgctggcgtttttccataggctccgcccccctgacgagcatcacaaaaatcgacgctcaagtcagaggtggcgaaacccgacaggactataaagataccaggcgtttccccctggaagctccctcgtgcgctctcctgttccgaccctgccgcttaccggatacctgtccgcctttctcccttcgggaagcgtggcgctttctcaatgctcacgctgtaggtatctcagttcggtgtaggtcgttcgctccaagctgggctgtgtgcacgaaccccccgttcagcccgaccgctgcgccttatccggtaactatcgtcttgagtccaacccggtaagacacgacttatcgccactggcagcagccactggtaacaggattagcagagcgaggtatgtaggcggtgctacagagttcttgaagtggtggcctaactacggctacactagaaggacagtatttggtatctgcgctctgctgaagccagttaccttcggaaaaagagttggtagctcttgatccggcaaacaaaccaccgctggtagcggtggtttttttgtttgcaagcagcagattacgcgcagaaaaaaaggatctcaagaagatcctttgatcttttctacggggtctgacgctcagtggaacgaaaactcacgttaagggattttggtcatgagattatcaaaaaggatcttcacctagatccttttggggtgggcgaagaactccagcatgagatccccgcgctggaggatcatccagccctgatagaaacagaagccactggagcacctcaaaaacaccatcatacactaaatcagtaagttggcagcatcacccgacgcactttgcgccgaataaatacctgtgacggaagatcacttcgcagaataaataaatcctggtgtccctgttgataccgggaagccctgggccaacttttggcgaaaatgagacgttgatcggcacgtaagaggttccaactttcaccataatgaaataagatcactaccgggcgtattttttgagttatcgagattttcaggagctgatagaaacagaagccactggagcacctcaaaaacaccatcatacactaaatcagtaagttggcagcatcacccgacgcactttgcgccgaataaatacctgtgacggaagatcacttcgcagaataaataaatcctggtgtccctgttgataccgggaagccctgggccaacttttggcgaaaatgagacgttgatcggcacgtaagaggttccaactttcaccataatgaaataagatcactaccgggcgtattttttgagttatcgagattttcaggagctctttggcatcgtctctcgcctgtcccctcagttcagtaatttcctgcatttgcctgtttccagtcggtagatattccacaaaacagcagggaagcagcgcttttccgctgcataaccctgcttcggggtcattatagcgattttttcggtatatccatcctttttcgcacgatatacaggattttgccaaagggttcgtgtagactttccttggtgtatccaacggcgtcagccgggcaggataggtgaagtaggcccacccgcgagcgggtgttccttcttcactgtcccttattcgcacctggcggtgctcaacgggaatcctgctctgcgaggctggccggctaccgccggcgtaacagatgagggcaagcggatggctgatgaaaccaagccaaccaggaagggcagcccacctatcaaggtgtactgccttccagacgaacgaagagcgattgaggaaaaggcggcggcggccggcatgagcctgtcggcctacctgctggccgtcggccagggctacaaaatcacgggcgtcgtggactatgagcacgtccgcgagggcgtcccggaaaacgattccgaagcccaacctttcatagaaggcggcggtggaatcgaaatctcgtgatggcaggttgggcgtcgcttggtcggtcatttcgaaaaaggttaggaatacggttagccatttgcctgcttttatatagttcantatgggattcacctttatgttgataagaaataaaagaaaatgccaataggatatcggcattttcttttgcgtttttatttgttaactgttaattgtccttgttcaaggatgctgtctttgacaacagatgttttcttgcctttgatgttcagcaggaagctcggcgcaaacgttgattgtttgtctgcgtagaatcctctgtttgtcatatagcttgtaatcacgacattgtttcctttcgcttgaggtacagcgaagtgtgagtaagtaaaggttacatcgttaggcggatcaagatccatttttaacacaaggccagttttgttcagcggcttgtatgggccagttaaagaattagaaacataaccaagcatgtaaatatcgttagacgtaatgccgtcaatcgtcatttttgatccgcgggagtcagtgaacaggtaccatttgccgttcattttaaagacgttcgcgcgttcaatttcatctgttactgtgttagatgcaatcagcggtttcatcacttttttcagtgtgtaatcatcgtttagctcaatcataccgagagcgccgtttgctaactcagccgtgcgttttttatcgctttgcagaagtttttgactttcttgacggaagaatgatgtgcttttgccatagtatgctttgttaaataaagattcttcgccttggtagccatcttcagttccagtgtttgcttcaaatactaagtatttgtggcctttatcttctacgtagtgaggatctctcagcgtatggttgtcgcctgagctgtagttgccttcatcgatgaactgctgtacattttgatacgtttttccgtcaccgtcaaagattgatttataatcctctacaccgttgatgttcaaagagctgtctgatgctgatacgttaacttgtgcagttgtcagtgtttgtttgccgtaatgtttaccggagaaatcagtgtagaataaacggatttttccgtcagatgtaaatgtggctgaacctgaccattcttgtgtttggtcttttaggatagaatcatttgcatcgaatttgtcgctgtctttaaagacgcggccagcgtttttccagctgtcaatagaagtttcgccgactttttgatagaacatgtaaatcgatgtgtcatccgcatttttaggatctccggctaatgcaaagacgatgtggtagccgtgatagtttgcgacagtgccgtcagcgttttgtaatggccagctgtcccaaacgtccaggccttttgcagaagagatatttttaattgtggacgaatcaaattcagaaacttgatatttttcatttttttgctgttcagggatttgcagcatatcatggcgtgtaatatgggaaatgccgtatgtttccttatatggcttttggttcgtttctttcgcaaacgcttgagttgcgcctcctgccagcagtgcggtagtaaaggttaatactgttgcttgttttgcaaactttttgatgttcatcgttcatgtctccttttttatgtactgtgttagcggtctgcttcttccagccctcctgtttgaagatggcaagttagttacgcacaataaaaaaagacctaaaatatgtaaggggtgacgccaaagtatacactttgccctttacacattttaggtcttgcctgctttatcagtaacaaacccgcgcgatttacttttcgacctcattctattagactctcgtttggattgcaactggtctattttcctcttttgtttgatagaaaatcataaaaggatttgcagactacgggcctaaagaactaaaaaatctatctgtttcttttcattctctgtattttttatagtttctgttgcatgggcataaagttgcctttttaatcacaattcagaaaatatcataatatctcatttcactaaataatagtgaacggcaggtatatgtgatgggttaaaaaggatcaccccagagtcccgctcagaagaactcgtcaagaaggcgatagaaggcgatgcgctgcgaatcgggagcggcgataccgtaaagcacgaggaagcggtcagcccattcgccgccaagctcttcagcaatatcacgggtagccaacgctatgtcctgatagcggtccgccacacccagccggccacagtcgatgaatccagaaaagcggccattttccaccatgatattcggcaagcaggcatcgccatgggtcacgacgagatcctcgccgtcgggcatccgcgccttgagcctggcgaacagttcggctggcgcgagcccctgatgctcttcgtccagatcatcctgatcgacaagaccggcttccatccgagtacgtgctcgctcgatgcgatgtttcgcttggtggtcgaatgggcaggtagccggatcaagcgtatgcagccgccgcattgcatcagccatgatggatactttctcggcaggagcaaggtgagatgacaggagatcctgccccggcacttcgcccaatagcagccagtcccttcccgcttcagtgacaacgtcgagacagctgcgcaaggaacgcccgtcgtggccagccacgatagccgcgctgcctcgtcttggagttcattcagggcaccggacaggtcggtcttgacaaaaagaaccgggcgcccctgcgctgacagccggaacacggcggcatcagagcagccgattgtctgttgtgcccagtcatagccgaatagcctctccacccaagcggccggagaacctgcgtgcaatccatcttgttcaatcatgcgaaacgatcctcatcctgtctcttgatcagatcttgatcccctgcgccatcagatccttggcggcaagaaagccatccagtttactttgcagggcttcccaaccttaccagagggcgccccagctggcaattccg